European Patent Application EP 4 285 929 A2, published December 6, 2023. Title: COMBINATION HBV THERAPY. Applicant: Vir Biotechnology, Inc. Application EP, filed August 7, 2023. The sequence listing filed with the application follows.

SEQUENCE LISTING (109 sequences)

SEQ ID NO: 1 - DNA, 3182 bp, Hepatitis B virus
  misc_feature 1..3182: note = NC_003977.2
  source 1..3182: mol_type = genomic DNA
aattccacaaccttccaccaaactctgcaagatcccagagtgagaggcctgtatttccctgctggtggctccagttcaggaacagtaaaccctgttctgactactgcctctcccttatcgtcaatcttctcgaggattggggaccctgcgctgaacatggagaacatcacatcaggattcctaggaccccttctcgtgttacaggcggggtttttcttgttgacaagaatcctcacaataccgcagagtctagactcgtggtggacttctctcaattttctagggggaactaccgtgtgtcttggccaaaattcgcagtccccaacctccaatcactcaccaacctcttgtcctccaacttgtcctggttatcgctggatgtgtctgcggcgttttatcatcttcctcttcatcctgctgctatgcctcatcttcttgttggttcttctggactatcaaggtatgttgcccgtttgtcctctaattccaggatcctcaacaaccagcacgggaccatgccggacctgcatgactactgctcaaggaacctctatgtatccctcctgttgctgtaccaaaccttcggacggaaattgcacctgtattcccatcccatcatcctgggctttcggaaaattcctatgggagtgggcctcagcccgtttctcctggctcagtttactagtgccatttgttcagtggttcgtagggctttcccccactgtttggctttcagttatatggatgatgtggtattgggggccaagtctgtacagcatcttgagtccctttttaccgctgttaccaattttcttttgtctttgggtatacatttaaaccctaacaaaacaaagagatggggttactctctaaattttatgggttatgtcattggatgttatgggtccttgccacaagaacacatcatacaaaaaatcaaagaatgttttagaaaacttcctattaacaggcctattgattggaaagtatgtcaacgaattgtgggtcttttgggttttgctgccccttttacacaatgtggttatcctgcgttgatgcctttgtatgcatgtattcaatctaagcaggctttcactttctcgccaacttacaaggcctttctgtgtaaacaatacctgaacctttaccccgttgcccggcaacggccaggtctgtgccaagtgtttgctgacgcaacccccactggctggggcttggtcatgggccatcagcgcatgcgtggaaccttttcggctcctctgccgatccatactgcggaactcctagccgcttgttttgctcgcagcaggtctggagcaaacattatcgggactgataactctgttgtcctatcccgcaaatatacatcgtttccatggctgctaggctgtgctgccaactggatcctgcgcgggacgtcctttgtttacgtcccgtcggcgctgaatcctgcggacgacccttctcggggtcgcttgggactctctcgtccccttctccgtctgccgttccgaccgaccacggggcgcacctctctttacgcggactccccgtctgtgccttctcatctgccggaccgtgtgcacttcgcttcacctctgcacgtcgcatggagaccaccgtgaacgcccaccaaatattgcccaaggtcttacataagaggactcttggactctcagcaatgtcaacgaccgaccttgaggcatacttcaaagactgtttgtttaaagactgggaggagttgggggaggagattaggttaaaggtctttgtactaggaggctgtaggcataaattggtctgcgcaccagcaccatgcaactttttcacctctgcctaatcatctcttgttcatgtcctactgttcaagcctccaagctgtgccttgggtggctttggggcatggacatcgacccttataaagaatttggagctactgtggagttactctcgtttttgccttctgacttctttccttcagtacgagatcttctagataccgcctcagctctgtatcgggaagccttagagtctcctgagcattgttcacctcaccatactgcactcaggcaagcaattctttgctggggggaactaatgactctagctacctgggtgggtgttaatttggaagatccagcgtctagagacctagtagtcagttatgtcaacactaatatgggcctaaagttcaggcaactcttgtggtttcacatttcttgtctcacttttggaagagaaacagttatagagtatttggtgtctttcggagtgtggattcgcactcctccagcttatagaccaccaaatgcccctatcctatcaacacttccggagactactgttgttagacgacgaggcaggtcccctagaagaagaactccctcgcctcgcagacgaaggtctcaatcgccgcgtcgcagaagatctcaatctcgggaatctcaatgttagtattccttggactcataaggtggggaactttactgggctttattcttctactgtacctgtctttaatcctcattggaaaacaccatcttttcctaatatacatttacaccaagacattatcaaaaaatgtgaacagtttgtaggcccactcacagttaatgagaaaagaagattgcaattgattatgcctgccaggttttatccaaaggttaccaaatatttaccattggataagggtattaaaccttattatccagaacatctagttaatcattacttccaaactagacactatttacacactctatggaaggcgggtatattatataagagagaaacaacacatagcgcctcattttgtgggtcaccatattcttgggaacaagatctacagcatggggcagaatctttccaccagcaatcctctgggattctttcccgaccaccagttggatccagccttcagagcaaacaccgcaaatccagattgggacttcaatcccaacaaggacacctggccagacgccaacaaggtaggagctggagcattcgggctgggtttcaccccaccgcacggaggccttttggggtggagccctcaggctcagggcatactacaaactttgccagcaaatccgcctcctgcctccaccaatcgccagtcaggaaggcagcctaccccgctgtctccacctttgagaaacactcatcctcaggccatgcagtgg

SEQ ID NO: 2 - DNA, 18 bp, Hepatitis B virus
  misc_feature 1..18: note = nucleotides 1579-1597 of NC_003977.2
  source 1..18: mol_type = genomic DNA
gtgtgcacttcgcttcac

SEQ ID NO: 3 - RNA, 19 nt, synthetic construct
  misc_feature 1..19: note = Synthetic sequence HBV02, sense strand
  source 1..19: mol_type = other RNA
gtgtgcacttcgcttcaca

SEQ ID NO: 4 - RNA, 21 nt, synthetic construct
  misc_feature 1..21: note = Synthetic sequence HBV02, antisense strand
  source 1..21: mol_type = other RNA
tgtgaagcgaagtgcacactt

SEQ ID NO: 5 - RNA, 19 nt, synthetic construct
  misc_feature 1..19: note = Synthetic oligonucleotide (HBV01, sense strand)
  source 1..19: mol_type = other RNA
gtgtgcacttcgcttcaca

SEQ ID NO: 6 - RNA, 21 nt, synthetic construct
  misc_feature 1..21: note = Synthetic oligonucleotide (HBV01, antisense strand)
  source 1..21: mol_type = other RNA
tgtgaagcgaagtgcacactt

SEQ ID NO: 7 - RNA, 19 nt, synthetic construct
  misc_feature 1..19: note = Synthetic oligonucleotide (HBV02, sense strand)
  source 1..19: mol_type = other RNA
gtgtgcacttcgcttcaca

SEQ ID NO: 8 - RNA, 21 nt, synthetic construct
  misc_feature 1..21: note = Synthetic oligonucleotide (HBV02, antisense strand)
  source 1..21: mol_type = other RNA
tgtgaagcgaagtgcacactt

SEQ ID NO: 9 - protein, 16 aa, synthetic construct
  REGION 1..16: note = Membrane translocation sequence-containing peptide RFGF
AAVALLPAVLLALLAP

SEQ ID NO: 10 - protein, 11 aa, synthetic construct
  REGION 1..11: note = Membrane translocation sequence-containing peptide RFGF analogue
AALLPVLLAAP

SEQ ID NO: 11 - protein, 13 aa, synthetic construct
  REGION 1..13: note = HIV Tat protein
GRKKRRQRRRPPQ

SEQ ID NO: 12 - protein, 15 aa, synthetic construct
  REGION 1..15: note = Drosophila Antennapedia protein
RQIKIWFQNRRMKWK

SEQ ID NO: 13 - protein, 226 aa, Hepatitis B virus
  REGION 1..226: note = HBsAg S domain
MENITSGFLGPLLVLQAGFFLLTRILTIPQSLDSWWTSLNFLGGTTVCLGQNSQSPTSNHSPTSCPPTCPGYRWMCLRRFIIFLFILLLCLIFLLVLLDYQGMLPVCPLIPGSSTTSTGPCRTCMTTAQGTSMYPSCCCTKPSDGNCTCIPIPSSWAFGKFLWEWASARFSWLSLLVPFVQWFVGLSPTVWLSVIWMMWYWGPSLYSILSPFLPLLPIFFCLWVYI

SEQ ID NO: 14 - protein, 72 aa, Hepatitis B virus
  REGION 1..72: note = J02203 (D, ayw3) HBsAg Antigenic Loop Sequence
QGMLPVCPLIPGSSTTSTGPCRTCMTTAQGTSMYPSCCCTKPSDGNCTCIPIPSSWAFGKFLWEWASARFSW

SEQ ID NO: 15 - protein, 72 aa, Hepatitis B virus
  REGION 1..72: note = FJ899792 (D, adw2) HBsAg Antigenic Loop Sequence
QGMLPVCPLIPGSSTTGTGPCRTCTTPAQGTSMYPSCCCTKPSDGNCTCIPIPSSWAFGKFLWEWASARFSW

SEQ ID NO: 16 - protein, 72 aa, Hepatitis B virus
  REGION 1..72: note = AM282986 (A) HBsAg Antigenic Loop Sequence
QGMLPVCPLIPGTTTTSTGPCKTCTTPAQGNSMFPSCCCTKPSDGNCTCIPIPSSWAFAKYLWEWASVRFSW

SEQ ID NO: 17 - protein, 72 aa, Hepatitis B virus
  REGION 1..72: note = D23678 (B1) HBsAg Antigenic Loop Sequence
QGMLPVCPLIPGSSTTSTGPCKTCTTPAQGTSMFPSCCCTKPTDGNCTCIPIPSSWAFAKYLWEWASVRFSW

SEQ ID NO: 18 - protein, 72 aa, Hepatitis B virus
  REGION 1..72: note = AB117758 (C1) HBsAg Antigenic Loop Sequence
QGMLPVCPLLPGTSTTSTGPCKTCTIPAQGTSMFPSCCCTKPSDGNCTCIPIPSSWAFARFLWEWASVRFSW

SEQ ID NO: 19 - protein, 74 aa, Hepatitis B virus
  REGION 1..74: note = AB205192(E) HBsAg Antigenic Loop Sequence
QGMLPVCPLIPGSSTTSTGPCRTCTTLAQGTSMFPSCCCSKPSDGNCTCIPIPSSWAFGKFLWEWASARFSWLS

SEQ ID NO: 20 - protein, 71 aa, Hepatitis B virus
  REGION 1..71: note = X69798 (F4) HBsAg Antigenic Loop Sequence
QGMLPVCPLLPGSTTTSTGPCTCTTLAQGTSMFPSCCCSKPSDGNCTCIPIPSSWALGKYLWEWASARFSW

SEQ ID NO: 21 - protein, 70 aa, Hepatitis B virus
  REGION 1..70: note = AF1 60501 (G) HBsAg Antigenic Loop Sequence
QGMLPVCPLIPGSSTTSTGPCTCTTPAQGNSMYPSCCCTPSDGNCTCIPIPSSWAFAKYLWEWASVRFSW

SEQ ID NO: 22 - protein, 72 aa, Hepatitis B virus
  REGION 1..72: note = AY090454 (H) HBsAg Antigenic Loop Sequence
QGMLPVCPLLPGSTTTSTGPCKTCTTLAQGTSMFPSCCCTKPSDGNCTCIPIPSSWAFGKYLWEWASARFSW

SEQ ID NO: 23 - protein, 72 aa, Hepatitis B virus
  REGION 1..72: note = AF241409 (I) HBsAg Antigenic Loop Sequence
QGMLPVCPLIPGSSTTSTGPCKTCTTPAQGNSMYPSCCCTKPSDGNCTCIPIPSSWAFAKYLWEWASARFSW

SEQ ID NO: 24 - protein, 72 aa, Hepatitis B virus
  REGION 1..72: note = AB486012 (J) HBsAg Antigenic Loop Sequence
QGMLPVCPLLPGSTTTSTGPCRTCTITAQGTSMFPSCCCTKPSDGNCTCIPIPSSWAFAKFLWEWASVRFSW

SEQ ID NO: 25 - protein, 72 aa, Hepatitis B virus
  REGION 1..72: note = HBsAg Y100C/P120T HBsAg Antigenic Loop Sequence
CQGMLPVCPLIPGSSTTGTGTCRTCTTPAQGTSMYPSCCCTKPSDGNCTCIPIPSSWAFGFLWEWASARFSW

SEQ ID NO: 26 - protein, 72 aa, Hepatitis B virus
  REGION 1..72: note = HBsAg P120T HBsAg Antigenic Loop Sequence
QGMLPVCPLIPGSSTTGTGTCRTCTTPAQGTSMYPSCCCTKPSDGNCTCIPIPSSWAFGKFLWEWASARFSW

SEQ ID NO: 27 - protein, 72 aa, Hepatitis B virus
  REGION 1..72: note = HBsAg P120T/S143L HBsAg Antigenic Loop Sequence
QGMLPVCPLIPGSSTTGTGTCRTCTTPAQGTSMYPSCCCTKPLDGNCTCIPIPSSWAFGKFLWEWASARFSW

SEQ ID NO: 28 - protein, 72 aa, Hepatitis B virus
  REGION 1..72: note = HBsAg C121 S HBsAg Antigenic Loop Sequence
QGMLPVCPLIPGSSTTGTGPSRTCTTPAQGTSMYPSCCCTKPSDGNCTCIPIPSSWAFGKFLWEWASARFSW

SEQ ID NO: 29 - protein, 72 aa, Hepatitis B virus
  REGION 1..72: note = HBsAg R122D HBsAg Antigenic Loop Sequence
QGMLPVCPLIPGSSTTGTGPCDTCTTPAQGTSMYPSCCCTKPSDGNCTCIPIPSSWAFGKFLWEWASARFSW

SEQ ID NO: 30 - protein, 71 aa, Hepatitis B virus
  REGION 1..71: note = HBsAg R122I HBsAg Antigenic Loop Sequence
QGMLPVCPLIPGSSTTGTGPCITCTTPAQGTSMYPSCCCTPSDGNCTCIPIPSSWAFGKFLWEWASARFSW

SEQ ID NO: 31 - protein, 72 aa, Hepatitis B virus
  REGION 1..72: note = HBsAg T123N HBsAg Antigenic Loop Sequence
QGMLPVCPLIPGSSTTGTGPCRNCTTPAQGTSMYPSCCCTKPSDGNCTCIPIPSSWAFGKFLWEWASARFSW

SEQ ID NO: 32 - protein, 72 aa, Hepatitis B virus
  REGION 1..72: note = HBsAg Q129H HBsAg Antigenic Loop Sequence
QGMLPVCPLIPGSSTTGTGPCRTCTTPAHGTSMYPSCCCTKPSDGNCTCIPIPSSWAFGKFLWEWASARFSW

SEQ ID NO: 33 - protein, 72 aa, Hepatitis B virus
  REGION 1..72: note = HBsAg Q129L HBsAg Antigenic Loop Sequence
QGMLPVCPLIPGSSTTGTGPCRTCTTPALGTSMYPSCCCTKPSDGNCTCIPIPSSWAFGKFLWEWASARFSW

SEQ ID NO: 34 - protein, 72 aa, Hepatitis B virus
  REGION 1..72: note = HBsAg M1 33H HBsAg Antigenic Loop Sequence
QGMLPVCPLIPGSSTTGTGPCRTCTTPAQGTSHYPSCCCTKPSDGNCTCIPIPSSWAFGKFLWEWASARFSW

SEQ ID NO: 35 - protein, 72 aa, Hepatitis B virus
  REGION 1..72: note = HBsAg M1 33L HBsAg Antigenic Loop Sequence
QGMLPVCPLIPGSSTTGTGPCRTCTTPAQGTSLYPSCCCTKPSDGNCTCIPIPSSWAFGKFLWEWASARFSW

SEQ ID NO: 36 - protein, 72 aa, Hepatitis B virus
  REGION 1..72: note = HBsAg M133T HBsAg Antigenic Loop Sequence
QGMLPVCPLIPGSSTTGTGPCRTCTTPAQGTSTYPSCCCTKPSDGNCTCIPIPSSWAFGKFLWEWASARFSW

SEQ ID NO: 37 - protein, 72 aa, Hepatitis B virus
  REGION 1..72: note = HBsAg K141 E HBsAg Antigenic Loop Sequence
QGMLPVCPLIPGSSTTGTGPCRTCTTPAQGTSMYPSCCCTEPSDGNCTCIPIPSSWAFGKFLWEWASARFSW

SEQ ID NO: 38 - protein, 72 aa, Hepatitis B virus
  REGION 1..72: note = HBsAg P142S HBsAg Antigenic Loop Sequence
QGMLPVCPLIPGSSTTGTGPCRTCTTPAQGTSMYPSCCCTKSSDGNCTCIPIPSSWAFGKFLWEWASARFSW

SEQ ID NO: 39 - protein, 72 aa, Hepatitis B virus
  REGION 1..72: note = HBsAg S143K HBsAg Antigenic Loop Sequence
QGMLPVCPLIPGSSTTGTGPCRTCTTPAQGTSMYPSCCCTKPKDGNCTCIPIPSSWAFGKFLWEWASARFSW

SEQ ID NO: 40 - protein, 71 aa, Hepatitis B virus
  REGION 1..71: note = HBsAg D144A HBsAg Antigenic Loop Sequence
QGMLPVCPLIPGSSTTGTGPCRTCTTPAQGTSMYPSCCCTPSAGNCTCIPIPSSWAFGKFLWEWASARFSW

SEQ ID NO: 41 - protein, 72 aa, Hepatitis B virus
  REGION 1..72: note = HBsAg G145R HBsAg Antigenic Loop Sequence
QGMLPVCPLIPGSSTTGTGPCRTCTTPAQGTSMYPSCCCTKPSDRNCTCIPIPSSWAFGKFLWEWASARFSW

SEQ ID NO: 42 - protein, 72 aa, Hepatitis B virus
  REGION 1..72: note = HBsAg N146A HBsAg Antigenic Loop Sequence
QGMLPVCPLIPGSSTTGTGPCRTCTTPAQGTSMYPSCCCTKPSDGACTCIPIPSSWAFGKFLWEWASARFSW

SEQ ID NO: 43 - protein, 226 aa, Hepatitis B virus
  REGION 1..226: note = HBsAg Genotype D S domain (Genbank accession no. FJ899792)
MENVTSGFLGPLLVLQAGFFLLTRILTIPQSLDSWWTSLNFLGGTTVCLGQNSQSPTSNHSPTSCPPTCPGYRWMCLRRFIIFLFILLLCLIFLLVLLDYQGMLPVCPLIPGSSTTGTGPCRTCTTPAQGTSMYPSCCCTKPSDGNCTCIPIPSSWAFGKFLWEWASARFSWLSLLVPFVQWFVGLSPTVWLSVIWMMWYWGPSLYSTLSPFLPLLPIFFCLWVYI

SEQ ID NO: 44 - protein, 8 aa, synthetic construct
  REGION 1..8: note = Synthetic sequence HBC34 CDRH1
GRIFRSFY

SEQ ID NO: 45 - protein, 7 aa, synthetic construct
  REGION 1..7: note = Synthetic sequence HBC34 short CDRH2
NQDGSEK

SEQ ID NO: 46 - protein, 8 aa, synthetic construct
  REGION 1..8: note = Synthetic sequence HBC34 long CDRH2
INQDGSEK

SEQ ID NO: 47 - protein, 12 aa, synthetic construct
  REGION 1..12: note = Synthetic sequence HBC34 CDRH3
AAWSGNSGGMDV

SEQ ID NO: 48 - protein, 6 aa, synthetic construct
  REGION 1..6: note = Synthetic sequence HBC34 CDRL1
KLGNKN

SEQ ID NO: 49 - skipped

SEQ ID NO: 50 - protein, 9 aa, synthetic construct
  REGION 1..9: note = Synthetic sequence HBC34 long CDRL2
VIYEVKYRP

SEQ ID NO: 51 - protein, 9 aa, synthetic construct
  REGION 1..9: note = Synthetic sequence HBC34 CDRL3
QTWDSTTVV

SEQ ID NO: 52 - protein, 9 aa, synthetic construct
  REGION 1..9: note = Synthetic sequence HBC34v35 CDRL3
QTFDSTTVV

SEQ ID NO: 53 - protein, 119 aa, synthetic construct
  REGION 1..119: note = Synthetic sequence HBC34 VH
ELQLVESGGGWVQPGGSQRLSCAASGRIFRSFYMSWVRQAPGKGLEWVATINQDGSEKLYVDSVKGRFTISRDNAKNSLFLQMNNLRVEDTAVYYCAAWSGNSGGMDVWGQGTTVSVSS

SEQ ID NO: 54 - protein, 119 aa, synthetic construct
  REGION 1..119: note = Synthetic sequence HBC34v31 VH
EVQLVESGGGLVQPGGSLRLSCAASGRIFRSFYMSWVRQAPGKGLEWVANINQDGSEKLYVDSVKGRFTISRDNAKNSLFLQMNNLRVEDTAVYYCAAWSGNSGGMDVWGQGTTVTVSS

SEQ ID NO: 55 - protein, 106 aa, synthetic construct
  REGION 1..106: note = Synthetic sequence HBC34 VL
SYELTQPPSVSVSPGQTVSIPCSGDKLGNKNVCWFQHKPGQSPVLVIYEVKYRPSGIPERFSGSNSGNTATLTISGTQAMDEAAYFCQTWDSTTVVFGGGTRLTVL

SEQ ID NO: 56 - protein, 106 aa, synthetic construct
  REGION 1..106: note = Synthetic sequence HBC34v7 VL
SYELTQPPSVSVSPGQTVSIPCSGDKLGNKNVCWFQHKPGQSPVLVIYEVKYRPSGIPERFSGSNSGNTATLTISGTQAMDEAAYFCQTFDSTTVVFGGGTRLTVL

SEQ ID NO: 57 - protein, 106 aa, synthetic construct
  REGION 1..106: note = Synthetic sequence HBC34v23 VL
SYELTQPPSVSVSPGQTASITCSGDKLGNKNACWYQQKPGQSPVLVIYEVKYRPSGIPERFSGSNSGNTATLTISGTQAMDEADYYCQTFDSTTVVFGGGTKLTVL

SEQ ID NO: 58 - protein, 106 aa, synthetic construct
  REGION 1..106: note = Synthetic sequence HBC34v34 VL
SYELTQPPSVSVSPGQTVSIPCSGDKLGNKNVSWFQHKPGQSPVLVIYEVKYRPSGIPERFSGSNSGNTATLTISGTQAMDEAAYFCQTFDSTTVVFGGGTRLTVL

SEQ ID NO: 59 - protein, 106 aa, synthetic construct
  REGION 1..106: note = Synthetic sequence HBC34v35 VL
SYELTQPPSVSVSPGQTVSIPCSGDKLGNKNVAWFQHKPGQSPVLVIYEVKYRPSGIPERFSGSNSGNTATLTISGTQAMDEAAYFCQTFDSTTVVFGGGTRLTVL

SEQ ID NO: 60 - protein, 106 aa, synthetic construct
  REGION 1..106: note = Synthetic sequence HBC34_LC40S VL
SYELTQPPSVSVSPGQTVSIPCSGDKLGNKNVSWFQHKPGQSPVLVIYEVKYRPSGIPERFSGSNSGNTATLTISGTQAMDEAAYFCQTWDSTTVVFGGGTRLTVL

SEQ ID NO: 61 - protein, 106 aa, synthetic construct
  REGION 1..106: note = Synthetic sequence HBC34_LC40A VL
SYELTQPPSVSVSPGQTVSIPCSGDKLGNKNVAWFQHKPGQSPVLVIYEVKYRPSGIPERFSGSNSGNTATLTISGTQAMDEAAYFCQTWDSTTVVFGGGTRLTVL

SEQ ID NO: 62 - protein, 106 aa, synthetic construct
  REGION 1..106: note = Synthetic sequence HBC34v23_LC40S VL
SYELTQPPSVSVSPGQTASITCSGDKLGNKNASWYQQKPGQSPVLVIYEVKYRPSGIPERFSGSNSGNTATLTISGTQAMDEADYYCQTFDSTTVVFGGGTKLTVL

SEQ ID NO: 63 - protein, 106 aa, synthetic construct
  REGION 1..106: note = Synthetic sequence HBC34v23_LC40A VL
SYELTQPPSVSVSPGQTASITCSGDKLGNKNAAWYQQKPGQSPVLVIYEVKYRPSGIPERFSGSNSGNTATLTISGTQAMDEADYYCQTFDSTTVVFGGGTKLTVL

SEQ ID NO: 64 - protein, 106 aa, synthetic construct; identical to SEQ ID NO: 60
  REGION 1..106: note = Synthetic sequence HBC34v31_LC40S VL

SEQ ID NO: 65 - protein, 106 aa, synthetic construct; identical to SEQ ID NO: 61
  REGION 1..106: note = Synthetic sequence HBC34v31_L C40A VL

SEQ ID NO: 66 - protein, 106 aa, synthetic construct; identical to SEQ ID NO: 58
  REGION 1..106: note = Synthetic sequence HBC34v32_LC40S VL

SEQ ID NO: 67 - protein, 106 aa, synthetic construct; identical to SEQ ID NO: 59
  REGION 1..106: note = Synthetic sequence HBC34v32_LC40A VL

SEQ ID NO: 68 - protein, 106 aa, synthetic construct; identical to SEQ ID NO: 62
  REGION 1..106: note = Synthetic sequence HBC34v33_LC40S VL

SEQ ID NO: 69 - protein, 106 aa, synthetic construct; identical to SEQ ID NO: 63
  REGION 1..106: note = Synthetic sequence HBC34v33_LC40A VL

SEQ ID NO: 70 - protein, 449 aa, synthetic construct
  REGION 1..449: note = Synthetic sequence HBC34v35 HC
ELQLVESGGGWVQPGGSQRLSCAASGRIFRSFYMSWVRQAPGKGLEWVATINQDGSEKLYVDSVKGRFTISRDNAKNSLFLQMNNLRVEDTAVYYCAAWSGNSGGMDVWGQGTTVSVSSASTKGPSVFPLAPSSKSTSGGTAALGCLVKDYFPEPVTVSWNSGALTSGVHTFPAVLQSSGLYSLSSVVTVPSSSLGTQTYICNVNHKPSNTKVDKKVEPKSCDKTHTCPPCPAPELLGGPSVFLFPPKPKDTLMISRTPEVTCVVVDVSHEDPEVKFNWYVDGVEVHNAKTKPREEQYNSTYRVVSVLTVLHQDWLNGKEYKCKVSNKALPAPIEKTISKAKGQPREPQVYTLPPSRDELTKNQVSLTCLVKGFYPSDIAVEWESNGQPENNYKTTPPVLDSDGSFFLYSKLTVDKSRWQQGNVFSCSVMHEALHNHYTQKSLSLSPGK

SEQ ID NO: 71 - protein, 449 aa, synthetic construct
  REGION 1..449: note = Synthetic sequence HBC34v35-MLNS-GAALIE (g1M17, 1) HC
ELQLVESGGGWVQPGGSQRLSCAASGRIFRSFYMSWVRQAPGKGLEWVATINQDGSEKLYVDSVKGRFTISRDNAKNSLFLQMNNLRVEDTAVYYCAAWSGNSGGMDVWGQGTTVSVSSASTKGPSVFPLAPSSKSTSGGTAALGCLVKDYFPEPVTVSWNSGALTSGVHTFPAVLQSSGLYSLSSVVTVPSSSLGTQTYICNVNHKPSNTKVDKKVEPKSCDKTHTCPPCPAPELLAGPSVFLFPPKPKDTLMISRTPEVTCVVVDVSHEDPEVKFNWYVDGVEVHNAKTKPREEQYNSTYRVVSVLTVLHQDWLNGKEYKCKVSNKALPLPEEKTISKAKGQPREPQVYTLPPSRDELTKNQVSLTCLVKGFYPSDIAVEWESNGQPENNYKTTPPVLDSDGSFFLYSKLTVDKSRWQQGNVFSCSVLHEALHSHYTQKSLSLSPGK

SEQ ID NO: 72 - protein, 449 aa, synthetic construct
  REGION 1..449: note = Synthetic sequence HBC34v35-MLNS HC
ELQLVESGGGWVQPGGSQRLSCAASGRIFRSFYMSWVRQAPGKGLEWVATINQDGSEKLYVDSVKGRFTISRDNAKNSLFLQMNNLRVEDTAVYYCAAWSGNSGGMDVWGQGTTVSVSSASTKGPSVFPLAPSSKSTSGGTAALGCLVKDYFPEPVTVSWNSGALTSGVHTFPAVLQSSGLYSLSSVVTVPSSSLGTQTYICNVNHKPSNTKVDKKVEPKSCDKTHTCPPCPAPELLGGPSVFLFPPKPKDTLMISRTPEVTCVVVDVSHEDPEVKFNWYVDGVEVHNAKTKPREEQYNSTYRVVSVLTVLHQDWLNGKEYKCKVSNKALPAPIEKTISKAKGQPREPQVYTLPPSRDELTKNQVSLTCLVKGFYPSDIAVEWESNGQPENNYKTTPPVLDSDGSFFLYSKLTVDKSRWQQGNVFSCSVLHEALHSHYTQKSLSLSPGK

SEQ ID NO: 73 - protein, 212 aa, synthetic construct
  REGION 1..212: note = Synthetic sequence HBC34v35 LC
SYELTQPPSVSVSPGQTVSIPCSGDKLGNKNVAWFQHKPGQSPVLVIYEVKYRPSGIPERFSGSNSGNTATLTISGTQAMDEAAYFCQTFDSTTVVFGGGTRLTVLGQPKAAPSVTLFPPSSEELQANKATLVCLISDFYPGAVTVAWKADSSPVKAGVETTTPSKQSNNKYAASSYLSLTPEQWKSHRSYSCQVTHEGSTVEKTVAPTECS

SEQ ID NO: 74 - protein, 212 aa, synthetic construct
  REGION 1..212: note = Synthetic sequence HBC34v34 LC
SYELTQPPSVSVSPGQTVSIPCSGDKLGNKNVSWFQHKPGQSPVLVIYEVKYRPSGIPERFSGSNSGNTATLTISGTQAMDEAAYFCQTFDSTTVVFGGGTRLTVLGQPKAAPSVTLFPPSSEELQANKATLVCLISDFYPGAVTVAWKADSSPVKAGVETTTPSKQSNNKYAASSYLSLTPEQWKSHRSYSCQVTHEGSTVEKTVAPTECS

SEQ ID NO: 75 - protein, 128 aa, synthetic construct
  REGION 1..128: note = Synthetic sequence HBC24 VH
EVQLLESGGGLVQPGGSLRLSCAASGSTFTKYAMSWVRQAPGKGLEWVASISGSVPGFGIDTYYADSVKGRFTISRDTSKNTLYLQMNSLRAEDTALYYCAKDVGVIGSYYYYAMDVWGQGTAVTVSS

SEQ ID NO: 76 - protein, 109 aa, synthetic construct
  REGION 1..109: note = Synthetic sequence HBC24 VL
EIVLTQSPGTLSLSPGERATLSCRASQGLSSSYLAWYQQKPGQAPRLLIYSASTRATGIPDRFSGSGSGTDFTLTISRLEPEDFAVYYCQQYAYSPRWTFGQGTKVEIK

SEQ ID NO: 77 - protein, 8 aa, synthetic construct
  REGION 1..8: note = Synthetic sequence HBC24 CDRH1
GSTFTKYA

SEQ ID NO: 78 - protein, 8 aa, synthetic construct
  REGION 1..8: note = Synthetic sequence HBC24 CDRH2
ISGSVPGF

SEQ ID NO: 79 - protein, 21 aa, synthetic construct
  REGION 1..21: note = Synthetic sequence HBC24 CDRH3
LYYCAKDVGVIGSYYYYAMDV

SEQ ID NO: 80 - protein, 7 aa, synthetic construct
  REGION 1..7: note = Synthetic sequence HBC24 CDRL1
QGLSSSY

SEQ ID NO: 81 - skipped

SEQ ID NO: 82 - protein, 10 aa, synthetic construct
  REGION 1..10: note = Synthetic sequence HBC24 CDRL3
QQYAYSPRWT

SEQ ID NO: 83 - protein, 212 aa, synthetic construct
  REGION 1..212: note = Synthetic sequence HBC34 LC
SYELTQPPSVSVSPGQTVSIPCSGDKLGNKNVCWFQHKPGQSPVLVIYEVKYRPSGIPERFSGSNSGNTATLTISGTQAMDEAAYFCQTWDSTTVVFGGGTRLTVLGQPKAAPSVTLFPPSSEELQANKATLVCLISDFYPGAVTVAWKADSSPVKAGVETTTPSKQSNNKYAASSYLSLTPEQWKSHRSYSCQVTHEGSTVEKTVAPTECS

SEQ ID NO: 84 - protein, 212 aa, synthetic construct
  REGION 1..212: note = Synthetic sequence HBC34v7 LC
SYELTQPPSVSVSPGQTVSIPCSGDKLGNKNVCWFQHKPGQSPVLVIYEVKYRPSGIPERFSGSNSGNTATLTISGTQAMDEAAYFCQTFDSTTVVFGGGTRLTVLGQPKAAPSVTLFPPSSEELQANKATLVCLISDFYPGAVTVAWKADSSPVKAGVETTTPSKQSNNKYAASSYLSLTPEQWKSHRSYSCQVTHEGSTVEKTVAPTECS

SEQ ID NO: 85 - protein, 212 aa, synthetic construct
  REGION 1..212: note = Synthetic sequence HBC34v23 LC
SYELTQPPSVSVSPGQTASITCSGDKLGNKNACWYQQKPGQSPVLVIYEVKYRPSGIPERFSGSNSGNTATLTISGTQAMDEADYYCQTFDSTTVVFGGGTKLTVLGQPKAAPSVTLFPPSSEELQANKATLVCLISDFYPGAVTVAWKADSSPVKAGVETTTPSKQSNNKYAASSYLSLTPEQWKSHRSYSCQVTHEGSTVEKTVAPTECS

SEQ ID NO: 86 - protein, 212 aa, synthetic construct
  REGION 1..212: note = Synthetic sequence HBC34_LC40S LC
SYELTQPPSVSVSPGQTVSIPCSGDKLGNKNVSWFQHKPGQSPVLVIYEVKYRPSGIPERFSGSNSGNTATLTISGTQAMDEAAYFCQTWDSTTVVFGGGTRLTVLGQPKAAPSVTLFPPSSEELQANKATLVCLISDFYPGAVTVAWKADSSPVKAGVETTTPSKQSNNKYAASSYLSLTPEQWKSHRSYSCQVTHEGSTVEKTVAPTECS

SEQ ID NO: 87 - protein, 212 aa, synthetic construct
  REGION 1..212: note = Synthetic sequence HBC34_LC40A LC
SYELTQPPSVSVSPGQTVSIPCSGDKLGNKNVAWFQHKPGQSPVLVIYEVKYRPSGIPERFSGSNSGNTATLTISGTQAMDEAAYFCQTWDSTTVVFGGGTRLTVLGQPKAAPSVTLFPPSSEELQANKATLVCLISDFYPGAVTVAWKADSSPVKAGVETTTPSKQSNNKYAASSYLSLTPEQWKSHRSYSCQVTHEGSTVEKTVAPTECS

SEQ ID NO: 88 - protein, 212 aa, synthetic construct
  REGION 1..212: note = Synthetic sequence HBC34v23_LC40S LC
SYELTQPPSVSVSPGQTASITCSGDKLGNKNASWYQQKPGQSPVLVIYEVKYRPSGIPERFSGSNSGNTATLTISGTQAMDEADYYCQTFDSTTVVFGGGTKLTVLGQPKAAPSVTLFPPSSEELQANKATLVCLISDFYPGAVTVAWKADSSPVKAGVETTTPSKQSNNKYAASSYLSLTPEQWKSHRSYSCQVTHEGSTVEKTVAPTECS

SEQ ID NO: 89 - protein, 212 aa, synthetic construct
  REGION 1..212: note = Synthetic sequence HBC34v23_LC40A LC
SYELTQPPSVSVSPGQTASITCSGDKLGNKNAAWYQQKPGQSPVLVIYEVKYRPSGIPERFSGSNSGNTATLTISGTQAMDEADYYCQTFDSTTVVFGGGTKLTVLGQPKAAPSVTLFPPSSEELQANKATLVCLISDFYPGAVTVAWKADSSPVKAGVETTTPSKQSNNKYAASSYLSLTPEQWKSHRSYSCQVTHEGSTVEKTVAPTECS

SEQ ID NO: 90 - protein, 212 aa, synthetic construct; identical to SEQ ID NO: 86
  REGION 1..212: note = Synthetic sequence HBC34v31_LC40S

SEQ ID NO: 91 - protein, 212 aa, synthetic construct; identical to SEQ ID NO: 87
  REGION 1..212: note = Synthetic sequence HBC34v31_LC40A LC

SEQ ID NO: 92 - protein, 212 aa, synthetic construct; identical to SEQ ID NO: 74
  REGION 1..212: note = Synthetic sequence HBC34v32_LC40S LC

SEQ ID NO: 93 - protein, 212 aa, synthetic construct; identical to SEQ ID NO: 73
  REGION 1..212: note = Synthetic sequence HBC34v32_LC40A LC

SEQ ID NO: 94 - protein, 212 aa, synthetic construct; identical to SEQ ID NO: 88
  REGION 1..212: note = Synthetic sequence HBC34v33_LC40S LC

SEQ ID NO: 95 - protein, 212 aa, synthetic construct; identical to SEQ ID NO: 89
  REGION 1..212: note = Synthetic sequence HBC34v33 _LC40A LC

SEQ ID NO: 96 - protein, 217 aa, Homo sapiens
  REGION 1..217: note = WT hIgG1 Fc
APELLGGPSVFLFPPKPKDTLMISRTPEVTCVVVDVSHEDPEVKFNWYVDGVEVHNAKTKPREEQYNSTYRVVSVLTVLHQDWLNGKEYKCKVSNKALPAPIEKTISKAKGQPREPQVYTLPPSRDELTKNQVSLTCLVKGFYPSDIAVEWESNGQPENNYKTTPPVLDSDGSFFLYSKLTVDKSRWQQGNVFSCSVMHEALHNHYTQKSLSLSPGK

SEQ ID NO: 97 - protein, 449 aa, synthetic construct
  REGION 1..449: note = Synthetic sequence HBC34+GAALIE HC
ELQLVESGGGWVQPGGSQRLSCAASGRIFRSFYMSWVRQAPGKGLEWVATINQDGSEKLYVDSVKGRFTISRDNAKNSLFLQMNNLRVEDTAVYYCAAWSGNSGGMDVWGQGTTVSVSSASTKGPSVFPLAPSSKSTSGGTAALGCLVKDYFPEPVTVSWNSGALTSGVHTFPAVLQSSGLYSLSSVVTVPSSSLGTQTYICNVNHKPSNTKVDKKVEPKSCDKTHTCPPCPAPELLAGPSVFLFPPKPKDTLMISRTPEVTCVVVDVSHEDPEVKFNWYVDGVEVHNAKTKPREEQYNSTYRVVSVLTVLHQDWLNGKEYKCKVSNKALPLPEEKTISKAKGQPREPQVYTLPPSRDELTKNQVSLTCLVKGFYPSDIAVEWESNGQPENNYKTTPPVLDSDGSFFLYSKLTVDKSRWQQGNVFSCSVMHEALHNHYTQKSLSLSPGK

SEQ ID NO: 98 - protein, 449 aa, synthetic construct
  REGION 1..449: note = Synthetic sequence HBC34v31+GAALIE HC
EVQLVESGGGLVQPGGSLRLSCAASGRIFRSFYMSWVRQAPGKGLEWVANINQDGSEKLYVDSVKGRFTISRDNAKNSLFLQMNNLRVEDTAVYYCAAWSGNSGGMDVWGQGTTVTVSSASTKGPSVFPLAPSSKSTSGGTAALGCLVKDYFPEPVTVSWNSGALTSGVHTFPAVLQSSGLYSLSSVVTVPSSSLGTQTYICNVNHKPSNTKVDKKVEPKSCDKTHTCPPCPAPELLAGPSVFLFPPKPKDTLMISRTPEVTCVVVDVSHEDPEVKFNWYVDGVEVHNAKTKPREEQYNSTYRVVSVLTVLHQDWLNGKEYKCKVSNKALPLPEEKTISKAKGQPREPQVYTLPPSRDELTKNQVSLTCLVKGFYPSDIAVEWESNGQPENNYKTTPPVLDSDGSFFLYSKLTVDKSRWQQGNVFSCSVMHEALHNHYTQKSLSLSPGK

SEQ ID NO: 99 - protein, 449 aa, synthetic construct
  REGION 1..449: note = Synthetic sequence murinized HBC34v7, BC34-v7-mu-IgG2a - HC
ELQLVESGGGWVQPGGSQRLSCAASGRIFRSFYMSWVRQAPGKGLEWVATINQDGSEKLYVDSVKGRFTISRDNAKNSLFLQMNNLRVEDTAVYYCAAWSGNSGGMDVWGQGTTVSVSSAKTTAPSVYPLAPVCGDTTGSSVTLGCLVKGYFPEPVTLTWNSGSLSSGVHTFPAVLQSDLYTLSSSVTVTSSTWPSQSITCNVAHPASSTKVDKKIEPRGPTIKPCPPCKCPAPNLLGGPSVFIFPPKIKDVLMISLSPIVTCVVVDVSEDDPDVQISWFVNNVEVHTAQTQTHREDYNSTLRVVSALPIQHQDWMSGKEFKCKVNNKDLPAPIERTISKPKGSVRAPQVYVLPPPEEEMTKKQVTLTCMVTDFMPEDIYVEWTNNGKTELNYKNTEPVLDSDGSYFMYSKLRVEKKNWVERNSYSCSVVHEGLHNHHTTKSFSRTPGK

SEQ ID NO: 100 - protein, 212 aa, synthetic construct
  REGION 1..212: note = Synthetic sequence murinized HBC34v7, BC34-v7-mu-IgG2a - LC
SYELTQPPSVSVSPGQTVSIPCSGDKLGNKNVCWFQHKPGQSPVLVIYEVKYRPSGIPERFSGSNSGNTATLTISGTQAMDEAAYFCQTFDSTTVVFGGGTRLTVLGQPKSSPSVTLFPPSSEELETNKATLVCTITDFYPGVVTVDWKVDGTPVTQGMETTQPSKQSNNKYMASSYLTLTARAWERHSSYSCQVTHEGHTVEKSLSRADCS

SEQ ID NO: 101 - protein, 449 aa, synthetic construct; identical to SEQ ID NO: 99
  REGION 1..449: note = Synthetic sequence murinized HBC34v35, HBC34-v35-mu-IgG2a - HC

SEQ ID NO: 102 - protein, 212 aa, synthetic construct
  REGION 1..212: note = Synthetic sequence murinized HBC34v35, HBC34-v35-mu-IgG2a - LC
SYELTQPPSVSVSPGQTVSIPCSGDKLGNKNVAWFQHKPGQSPVLVIYEVKYRPSGIPERFSGSNSGNTATLTISGTQAMDEAAYFCQTFDSTTVVFGGGTRLTVLGQPKSSPSVTLFPPSSEELETNKATLVCTITDFYPGVVTVDWKVDGTPVTQGMETTQPSKQSNNKYMASSYLTLTARAWERHSSYSCQVTHEGHTVEKSLSRADCS

SEQ ID NO: 103 - protein, 458 aa, synthetic construct
  REGION 1..458: note = Synthetic sequence murinized HBC24, HBC24-mu-IgG2a - HC
EVQLLESGGGLVQPGGSLRLSCAASGSTFTKYAMSWVRQAPGKGLEWVASISGSVPGFGIDTYYADSVKGRFTISRDTSKNTLYLQMNSLRAEDTALYYCAKDVGVIGSYYYYAMDVWGQGTAVTVSSAKTTAPSVYPLAPVCGDTTGSSVTLGCLVKGYFPEPVTLTWNSGSLSSGVHTFPAVLQSDLYTLSSSVTVTSSTWPSQSITCNVAHPASSTKVDKKIEPRGPTIKPCPPCKCPAPNLLGGPSVFIFPPKIKDVLMISLSPIVTCVVVDVSEDDPDVQISWFVNNVEVHTAQTQTHREDYNSTLRVVSALPIQHQDWMSGKEFKCKVNNKDLPAPIERTISKPKGSVRAPQVYVLPPPEEEMTKKQVTLTCMVTDFMPEDIYVEWTNNGKTELNYKNTEPVLDSDGSYFMYSKLRVEKKNWVERNSYSCSVVHEGLHNHHTTKSFSRTPGK

SEQ ID NO: 104 - protein, 215 aa, synthetic construct
  REGION 1..215: note = Synthetic sequence murinized HBC24, HBC24-mu-IgG2a - LC
EIVLTQSPGTLSLSPGERATLSCRASQGLSSSYLAWYQQKPGQAPRLLIYSASTRATGIPDRFSGSGSGTDFTLTISRLEPEDFAVYYCQQYAYSPRWTFGQGTKVEIKADAAPTVSIFPPSSEQLTSGGASVVCFLNNFYPKDINVKWKIDGSERQNGVLNSWTDQDSKDSTYSMSSTLTLTKDEYERHNSYTCEATHKTSTSPIVKSFNRNEC

SEQ ID NO: 105 - protein, 19 aa, synthetic construct
  REGION 1..19: note = Synthetic sequence chimeric hinge
ESKYGPPCPPCPAPPVAGP

SEQ ID NO: 106 - RNA, 21 nt, synthetic construct
  misc_feature 1..21: note = Synthetic sequence siRNA3 sense strand
  source 1..21: mol_type = other RNA
ggtggacttctctcaatttta

SEQ ID NO: 107 - RNA, 23 nt, synthetic construct
  misc_feature 1..23: note = Synthetic sequence siRNA3 antisense strand
  source 1..23: mol_type = other RNA
taaaattgagagaagtccaccac

SEQ ID NO: 108 - RNA, 21 nt, synthetic construct
  misc_feature 1..21: note = Synthetic oligonucleotide (siRNA3 sense strand)
  source 1..21: mol_type = other RNA
ggtggacttctctcaatttta

SEQ ID NO: 109 - RNA, 23 nt, synthetic construct
  misc_feature 1..23: note = Synthetic oligonucleotide (siRNA3 antisense strand)
  source 1..23: mol_type = other RNA
taaaattgagagaagtccaccac